European Patent Application EP 4 345 168 A2, published April 3, 2024. Title: Methods for preparing DNA reference material and controls. Applicant: LGC Clinical Diagnostics, Inc. The sequence listing filed with the application follows.

SEQUENCE LISTING (11 sequences)

SEQ ID NO: 1 - DNA, 33 bp, synthetic construct
  misc_feature 1..33: note = Description of Artificial Sequence: Synthetic oligonucleotide
  source 1..33: mol_type = other DNA
gaagagccctatatgggatgatctgaccgtcgt

SEQ ID NO: 2 - DNA, 34 bp, synthetic construct
  misc_feature 1..34: note = Description of Artificial Sequence: Synthetic oligonucleotide
  source 1..34: mol_type = other DNA
tgattttgcctggcgtgttgtatagggctcttct

SEQ ID NO: 3 - DNA, 20 bp, synthetic construct
  misc_feature 1..20: note = Description of Artificial Sequence: Synthetic primer
  source 1..20: mol_type = other DNA
acgacggtcagatcatccca

SEQ ID NO: 4 - DNA, 20 bp, synthetic construct
  misc_feature 1..20: note = Description of Artificial Sequence: Synthetic primer
  source 1..20: mol_type = other DNA
tgattttgcctggcgtgttg

SEQ ID NO: 5 - DNA, 20 bp, synthetic construct
  misc_feature 1..20: note = Description of Artificial Sequence: Synthetic primer
  source 1..20: mol_type = other DNA
acgacggtcagatcatccca

SEQ ID NO: 6 - DNA, 20 bp, synthetic construct
  misc_feature 1..20: note = Description of Artificial Sequence: Synthetic primer
  source 1..20: mol_type = other DNA
tgattttgcctggcgtgttg

SEQ ID NO: 7 - DNA, 16 bp, Homo sapiens
  source 1..16: mol_type = other DNA
ggaattaagagaagca

SEQ ID NO: 8-9 - skipped (2 entries)

SEQ ID NO: 10 - protein, 5 aa, Homo sapiens
ELREA

SEQ ID NO: 11 - protein, 6 aa, synthetic construct
  REGION 1..6: note = Description of Artificial Sequence: Synthetic peptide
AYVMAG